European Patent Specification EP 4 043 560 B1, published August 13, 2025. Title: Group of Glycosyltransferases and Use Thereof. Applicant: SHANGHAI INSTITUTES FOR BIOLOGICAL SCIENCES, CHINESE ACADEMY OF SCIENCES. The sequence listing filed with the application follows.

SEQUENCE LISTING (70 sequences)

SEQ ID NO: 1 - DNA, 1425 bp, Panax ginseng
  misc_feature: gGT25
atgaagtcagaattgatattcttgcccgccccggccatcggacacctcgtgggaatggtggagatggctaaactcttcatcagtcgacatgaaaacctctcggtcaccgtcctcatcgcgaaattctacatggatacgggggtagacaactacaataaatcactcttaacaaaccctaccccgcgtctcacaattgtaaatctcccggaaaccgacccccaaaactatatgctcaaaccacgccatgccatctttcctagcgtcatcgagactcagaagacacacgtgcgagacataatatcaggcatgactcagtccgagtcgactcgggtcgttggtttgctggctgaccttttgttcatcaacattatggacattgccaatgagttcaatgttccaacttatgtatactcccctgccggagccggtcatcttggcctcgcgttccatctccagacactcaacgacaaaaagcaagatgtgaccgagttcaggaactcggacactgagttattggtaccgagttttgcaaacccggttcccgccgaggtcttgccgtcgatgtatgtggataaagaaggtgggtatgattatttgttttcattgttccggaggtgcagagagtcaaaggcaattattattaacacgtttgaggagctggaaccctatgcgatcaattccctccggatggatagtatgatccctccgatctacccggtgggacccatactaaatctcaacggtgatggccaaaactccgatgaggctgctgtgatccttggttggttagatgatcaaccaccttcatctgtggtgtttttgtgctttggtagctatggaagctttcaagaaaaccaggtgaaggagattgcaatgggtctagagcgcagtgggcatcgcttcttgtggtccttgcgtccgtctatccctaaaggcgagacaaagcttcagcttaaatactcaaatttgaaagaaattctcccagtaggattcttggacaggacatcatgcgtcggaaaagtgattggatgggccccgcaagtggccgtgctcggacatgagtcagtcggagggttcctgtctcattgcggttggaattcgacattggagagtgtttggtgtggggtgcccgttgcaacatggccaatgtatggtgagcaacaactcaatgcttttgagatggttaaggagttaggtattgcggtggaaattgaggtggactataagaaagattattttaacatgaagaatgattttattgttagggcagaagaaatcgagacaaaaataaagaagttgatgatggatgaaaataatagtgaaataagaaagaaggtaaaggaaatgaaagaaaagagtagggctgcaatgtctgagaatggatcatcttataattcattggcgaagctatttgaggaaattatg

SEQ ID NO: 2 - protein, 475 aa, Panax ginseng
  misc_feature: gGT25
MKSELIFLPAPAIGHLVGMVEMAKLFISRHENLSVTVLIAKFYMDTGVDNYNKSLLTNPTPRLTIVNLPETDPQNYMLKPRHAIFPSVIETQKTHVRDIISGMTQSESTRVVGLLADLLFINIMDIANEFNVPTYVYSPAGAGHLGLAFHLQTLNDKKQDVTEFRNSDTELLVPSFANPVPAEVLPSMYVDKEGGYDYLFSLFRRCRESKAIIINTFEELEPYAINSLRMDSMIPPIYPVGPILNLNGDGQNSDEAAVILGWLDDQPPSSVVFLCFGSYGSFQENQVKEIAMGLERSGHRFLWSLRPSIPKGETKLQLKYSNLKEILPVGFLDRTSCVGKVIGWAPQVAVLGHESVGGFLSHCGWNSTLESVWCGVPVATWPMYGEQQLNAFEMVKELGIAVEIEVDYKKDYFNMKNDFIVRAEEIETKIKKLMMDENNSEIRKKVKEMKEKSRAAMSENGSSYNSLAKLFEEIM

SEQ ID NO: 3 - DNA, 1431 bp, Panax ginseng
  misc_feature: gGT13
atgggagcggagctcatcttaatcccttctccgggagttggtcatctggtatctactgttgagattgcaaagctcctcatcagtcgagatgaacggctttccatcacagtccttgtaatgaagttctcgcatgacactggtgtgactgcctacactcggtcattgcagaaagatgctcctaaccgcatagtctttgtggaccttcctcagaacgagtctcttatctcatcgcccaagtctttctttactagcttcatcgagagtcagacgagtccggttagagattctgtcagacaaattgtgagtcggtctgattctaataagctcgctggcttcgtcatcgacatgttctgcaccccaatgatagacgtggcaaatgaatttggagtcccaacctatgtgttcttcacttcaggtgctgcatttcttggcctccagttttaccatctgagtctcagtgatgaacataaccaggaccttaccgagtataaggacacggatgttgagttatctatcccgagtttcatcaacccagtgcccgctaaggttttgccttcggtgattctgaacaaggaaggatcgaccatgctccaatctatttcccgaaggtttaaagaagccaaggccattctagtcaacacgttcgcggagctggaaccacatgccattaaggcccttggtgataactgcaagatccctcctatctatcccgtgggacccataatcaacctcaagaacaaggagggaacaacccaaaaccatagttctgaagatggtatcattagctggttggacaatcagccaccatcttcggtagtgtttttgtgctttgggagctttgggagctttgatgaaggccaagtcagggagatagcaaacggattggagcagagtggacagcgattcttgtggtctctacgccggcggccagaaaaaatggaattgcctaaagactatgagaatcccgaagaagtgttgccagaaggattcatagaacgaacatcagggatggggaaggtgatcggatgggcgccacaaacggcgattctttcccaccctgctgtgggaggattcgtgtctcattgtggatggaattctacattggagagtatatggtgtggggttccaatggctacttggcctatatatgcagagcagcaaatcaatgcgtttgagttggtgaaggagttgggaatggctgtggagatcaaaatggattacagagaagattatatttttgcacctgaaaataatttagttgtgaccgcagaccagatagagaaaggaatgcgatgtctgatgatggatggagagagtgaaatgaggaagaaggtggaagagatgaaagagaagagcagaatggccatggtgaagggcgggtcttcttacatttcactcgggcattttattgaggatgtcatgcgtaattaa

SEQ ID NO: 4 - protein, 476 aa, Panax ginseng
  misc_feature: gGT13
MGAELILIPSPGVGHLVSTVEIAKLLISRDERLSITVLVMKFSHDTGVTAYTRSLQKDAPNRIVFVDLPQNESLISSPKSFFTSFIESQTSPVRDSVRQIVSRSDSNKLAGFVIDMFCTPMIDVANEFGVPTYVFFTSGAAFLGLQFYHLSLSDEHNQDLTEYKDTDVELSIPSFINPVPAKVLPSVILNKEGSTMLQSISRRFKEAKAILVNTFAELEPHAIKALGDNCKIPPIYPVGPIINLKNKEGTTQNHSSEDGIISWLDNQPPSSVVFLCFGSFGSFDEGQVREIANGLEQSGQRFLWSLRRRPEKMELPKDYENPEEVLPEGFIERTSGMGKVIGWAPQTAILSHPAVGGFVSHCGWNSTLESIWCGVPMATWPIYAEQQINAFELVKELGMAVEIKMDYREDYIFAPENNLVVTADQIEKGMRCLMMDGESEMRKKVEEMKEKSRMAMVKGGSSYISLGHFIEDVMRN

SEQ ID NO: 5 - DNA, 1353 bp, Panax ginseng
  misc_feature: gGT30
atggcaacccaaaaatgtttccgtgtcctcgtgttcccatggttagctcatggtcacatctcccccttcctagaactagccagaaaacttatagaaaaaggaaactttttcatttacttctgctccactcctataaatctcatctccataaagaaaaaacttagtggtgatgatcatcaaaattacaccaagtcaatacaactagtggaacacaatctaccgaccttacctcaacttcctcctcactaccacaccaccgacggcctcccaccaaatctcaatcctacccttcgaaaggcatttgaaatgtcaaaactatccttccccaacaccctaaacactttgaaaccagatctactcatttgtgatgacttatttcaatggccagaaatagtagcttcatcacatggtgttccggttgttcggttccaaacatgcagcgtgacagccgctagttttctagctcatatttttacgaacccagacgttacatacccttttccagccatttatcttcatgagtatgaaactgatcagatcaggcgttgcgttgacgcggtttttgaaagcggcagagaagaatctcgcaacctgttggttgtcaacacgtctaaagcgatcgaggaaaaatatttttattattattctctacttcggggtaacaccaaaattatgccagttggtccgcttattcagcaagccccaaatggcgacgaggatatgaaggtcatcgaatggcttgacaagaaggatccgtgttcaaccgtgttcgtgtcctttgggagcgagtattttatgcaaaaagaagaggttgaagagatggctcatggtttagagcttagcaacgtcaatttcatctgggtttttagggctccggtgggagcggaaaaggttaagctgccgttagggtttgttgagagggttggggggaggggaattgttatggaggggtgggccccacaggcaaggattttgggacattcaagtattggtgggtttgtgagtcattgtgggtggaattctgtgttggaaactataaattttggtgttccaataatagggatgccaatgaaatttgagcagcctatgaatgctaggcttctatctgaacttggtgtttgtgttgaaattgtgggggacgaaactaggaggtttggaagagaagaggtaggaaatgtaataagagaagtggttggtgggaagataggggacgatttgagaaggaaagtgaaagaacttggagcaaagataaaggaaaaacaagaggaagagatggatgatgtgcttgatgaattagtacaaatttgtaacaagaaaaaacggactgttgtacatcatcatcatcatcattga

SEQ ID NO: 6 - protein, 450 aa, Panax ginseng
  misc_feature: gGT30
MATQKCFRVLVFPWLAHGHISPFLELARKLIEKGNFFIYFCSTPINLISIKKKLSGDDHQNYTKSIQLVEHNLPTLPQLPPHYHTTDGLPPNLNPTLRKAFEMSKLSFPNTLNTLKPDLLICDDLFQWPEIVASSHGVPVVRFQTCSVTAASFLAHIFTNPDVTYPFPAIYLHEYETDQIRRCVDAVFESGREESRNLLVVNTSKAIEEKYFYYYSLLRGNTKIMPVGPLIQQAPNGDEDMKVIEWLDKKDPCSTVFVSFGSEYFMQKEEVEEMAHGLELSNVNFIWVFRAPVGAEKVKLPLGFVERVGGRGIVMEGWAPQARILGHSSIGGFVSHCGWNSVLETINFGVPIIGMPMKFEQPMNARLLSELGVCVEIVGDETRRFGREEVGNVIREVVGGKIGDDLRRKVKELGAKIKEKQEEEMDDVLDELVQICNKKKRTVVHHHHHH

SEQ ID NO: 7 - DNA, 26 bp, Panax ginseng
ccaagttcattcaagatgaagtcaga

SEQ ID NO: 8 - DNA, 28 bp, Artificial sequence
cataatttcctcaaatagcttcgccaat

SEQ ID NO: 9 - DNA, 24 bp, Artificial sequence
actggagcagttgcaacatacaaa

SEQ ID NO: 10 - DNA, 24 bp, Artificial sequence
tcatttatgcgctttcctggatgt

SEQ ID NO: 11 - DNA, 21 bp, Artificial sequence
acgagggtggttttaatggca

SEQ ID NO: 12 - DNA, 27 bp, Artificial sequence
acaccattcataatcatacaacagtcc

SEQ ID NO: 13 - DNA, 29 bp, Artificial sequence
atatggtaccatggcagtagccggcgctg

SEQ ID NO: 14 - DNA, 57 bp, Artificial sequence
gcgctctagattaatgatgatgatgatgatgttttattatatgttttttggggtcgc

SEQ ID NO: 15 - DNA, 1428 bp, Panax ginseng
  misc_feature: gGT25-1
atgaagtcagaattgatattcttgcccgccccggccatcggacacctcgtgggaatggtggagatggctaaactcttcatcagtcgacatgaaaacctctcggtcaccgtcctcatcgcgaaattctacatggatacgggggtagacaactacaataaatcactcttaacaaaccctaccccgcgtctcacaattgtaaatctcccggaaaccgacccccaaaactatatgctcaaaccacgccatgccatctttcctagcgtcatcgagactcagaagacacacgtgcgagacataatatcaggcatgactcagtccgagtcgactcgggtcgttggtttgctggctgaccttttgttcatcaacattatggacattgccaatgagttcaatgttccaacttatgtatactcccctgccggagccggtcatcttggcctcgcgttccatctccagacactcaacgacaaaaagcaagatgtgaccgagttcaggaactcggacactgagttattggtaccgagttttgcaaacccggttcccgccgaggtcttgccgtcgatgtatgtggataaagaaggtgggtatgattatttgttttcattgttccggaggtgcagagagtcaaaggcaattattattaacacgtttgaggagctggaaccctatgcgatcaattccctccggatggatagtatgatccctccgatctacccggtgggacccatactaaatctcaacggtgatggccaaaactccgatgaggctgctgtgatccttggttggttagatgatcaaccaccttcatctgtggtgtttttgtgctttggtagctatggaacctttcaagaaaaccaggtgaaggagattgcaatgggtctagagcgcagtgggcatcgcttcttgtggtccttgcgtccgtctatccctaaaggcgagacaaagcttcagcttaaatactcaaatttggaagaaattctcccagtcggattcttggacaggacatcatgcgtcggaaaagttattggatgggccccgcaagtggcggtgctcggacacgaggcagtcggagggttcctgtctcattgtggttggaattcgacattagagagtgtgtggtgtggcgtgcccgtcgcaacatggccaatgtacggcgagcaacaactcaatgcttttgagatggttaaggagttaggtattgcggtggaaattgaggtggactataagaatgaatattttaacatgaataatgattttattgttagggcagaagaaatcgagacgaaaataaagaagttgatgatggatgaaaagaatagtgaaataaggaagaaggtaaaggaaatgaaagaaaagagtaggcttgcaatgtctgagaatggatcatcttataattcattggcgaagctatttgaggaaatcatgtaa

SEQ ID NO: 16 - protein, 475 aa, Panax ginseng
  misc_feature: gGT25-1
MKSELIFLPAPAIGHLVGMVEMAKLFISRHENLSVTVLIAKFYMDTGVDNYNKSLLTNPTPRLTIVNLPETDPQNYMLKPRHAIFPSVIETQKTHVRDIISGMTQSESTRVVGLLADLLFINIMDIANEFNVPTYVYSPAGAGHLGLAFHLQTLNDKKQDVTEFRNSDTELLVPSFANPVPAEVLPSMYVDKEGGYDYLFSLFRRCRESKAIIINTFEELEPYAINSLRMDSMIPPIYPVGPILNLNGDGQNSDEAAVILGWLDDQPPSSVVFLCFGSYGTFQENQVKEIAMGLERSGHRFLWSLRPSIPKGETKLQLKYSNLEEILPVGFLDRTSCVGKVIGWAPQVAVLGHEAVGGFLSHCGWNSTLESVWCGVPVATWPMYGEQQLNAFEMVKELGIAVEIEVDYKNEYFNMNNDFIVRAEEIETKIKKLMMDEKNSEIRKKVKEMKEKSRLAMSENGSSYNSLAKLFEEIM

SEQ ID NO: 17 - DNA, 1428 bp, Panax ginseng
  misc_feature: gGT25-3
atgaagtcagaattgatattcttgcccgccccggccatcggacacctcgtgggaatggtggagatggctaaactcttcatcagtcgacatgaaaatctctcggtcaccgtcctcatcgcgaaattctacatggatacgggggtagacaactacaataaatcactcttaacaaaccctaccccgcgtctcacaattgtaaatctcccggaaaccgacccccaaaactatatgctcaaaccacgccacgccatctttcctagcgtcatcgagactcagaagacacacgtgcgagacataatatccggtatgactcagtccgagtcgactcaggtcgttggtttgctggctgaccttttgttcatcaacatcatggacattgccaatgagttcaatgttccaacttatgtatactcccctgccggagccggtcatcttggcctcgcgttccatctccagacactcaacgacaaaaaacaagatgtgaccgagttcaggaactcggatactgagttattggtaccgagttttgcaaacccggttcccgccgaggtcttgccgtcgatgtatgtggataaagaaggtgggtatgattatctgttttcattgttccggaggtgcagagagtcaaaggcaattattattaacacgtttgaggagctggaaccctatgcgatcaattccctccggatggatagtatgatccctccgatctacccggtgggacccatactaaatctcaacggtgatggccaaaactccgatgaggctgctgtgatccttggttggttagatgatcaaccaccttcatctgtggtgtttttgtgctttggtagctatggaagctttcaagaaaaccaggtgaaggagattgcaatgggtctagagcgcagtgggcatcgcttcttgtggtccttgcgtccgtctatccctaaaggcgagacaaagcttcagcttaaatactcaaatttgaaagaaattctcccagtaggattcttggacaggacatcatgcgtcggaaaagtgattggatgggccccgcaagtggccgtgctcggacatgagtcagtcggagggttcctgtctcattgcggttggaattcgacattggagagtgtttggtgtggggtgcccgttgcaacatggccaatgtatggtgagcaacaactcaatgcttttgagatggttaaggagttaggtattgcggtggaaattgaggtggactataagaaagattattttaacatgaagaatgattttattgttagggcagaagaaatcgagacaaaaataaagaagttgatgatggatgaaaataatagtgaaataagaaagaaggtaaaggaaatgaaagaaaagagtagggctgcaatgtctgagaatggatcatcttataattcattggcgaagctatttgaggaaattatgtaa

SEQ ID NO: 18 - protein, 475 aa, Panax ginseng
  misc_feature: gGT25-3
MKSELIFLPAPAIGHLVGMVEMAKLFISRHENLSVTVLIAKFYMDTGVDNYNKSLLTNPTPRLTIVNLPETDPQNYMLKPRHAIFPSVIETQKTHVRDIISGMTQSESTQVVGLLADLLFINIMDIANEFNVPTYVYSPAGAGHLGLAFHLQTLNDKKQDVTEFRNSDTELLVPSFANPVPAEVLPSMYVDKEGGYDYLFSLFRRCRESKAIIINTFEELEPYAINSLRMDSMIPPIYPVGPILNLNGDGQNSDEAAVILGWLDDQPPSSVVFLCFGSYGSFQENQVKEIAMGLERSGHRFLWSLRPSIPKGETKLQLKYSNLKEILPVGFLDRTSCVGKVIGWAPQVAVLGHESVGGFLSHCGWNSTLESVWCGVPVATWPMYGEQQLNAFEMVKELGIAVEIEVDYKKDYFNMKNDFIVRAEEIETKIKKLMMDENNSEIRKKVKEMKEKSRAAMSENGSSYNSLAKLFEEIM

SEQ ID NO: 19 - DNA, 1419 bp, Panax ginseng
  misc_feature: gGT25-5
atgaagtcagaattgatattcgtgcccgtcccggccttcgggcacctcgtggggatggtggagatggctaaacttttcatcagtcgacacgaaaacctatcagtcaccgtcctcatttcgaaatttttcattgatacggggatagacaactacaataaatcactcttagcgaaacctaccccgcgtctcacaattataaatctcccggaaatcgatccccaaaaatatttgctcaaaccacgttgcgccatctttccttccctcatcgagaatcagaagacacacgtgcgagacgtaatgtcccgcatgactcagtccgagtcgactcgggtcgttggtttgctggcagacattttgttcgtcgacatcttcgacattgccgatgagttcaatgttccaacttatgtatactcccctgccggagccggttttcttggcctcgcgttccatctccagacactcaacgacgacaaaaagcaagatgtgaccgagttcaggaattcggacactgagttattggtaccgagttttgcaaacccggtccccgccgagttcttgccgtcgatatttttggaaaaagatggtaggcatgatgttttgttatcattgtactggaggtgcagggaggcaaagggaattattgttaacacgtttgaggagctggaaccctatgcgatcaattccctccggatggatagtatgatccctccgatctacccggtgggacccatactaaatctcaacggtgagggacaaaactccgatgaggctgctgtgatccttggttggttagatgatcaaccaccttcatctgtggtgtttttgtgctttggtagctttggaagctttccagaaaaccaggtgaaggagattgcaatgggtttagagcgcagcgggcatcgcttcttgtggtccttgcgtccgtgtatctctgaaggtgagacaacgcttcaacttaaatactcaaatttggaacttccggccggattcttggataggacatcatgcgtcggaaaagtgattggatgggccccacaaatggccatcctagcacacgaggcagtcggagggttcgtgtctcattgtggttggaattcggtactagagagtgtgtggtatggcatgcctgtcgcaacatggccaatgtacggtgagcaacaactcaacgcttttgagatggttaaggagttgggtcttgcggtggaaattgaggtggactataggaatgaatataacaagtctgattttattgttaaggctgacgaaattgagacaaaaataaagaagttgatgatggatggaaagaatagtaaaataaggaagaaggtaaaggaaatgaaagaaaagagtagggttgccatgtcggagaatgggtcatcttatacttcattggcgaagctatttgaggaaattatgtaa

SEQ ID NO: 20 - protein, 472 aa, Panax ginseng
  misc_feature: gGT25-5
MKSELIFVPVPAFGHLVGMVEMAKLFISRHENLSVTVLISKFFIDTGIDNYNKSLLAKPTPRLTIINLPEIDPQKYLLKPRCAIFPSLIENQKTHVRDVMSRMTQSESTRVVGLLADILFVDIFDIADEFNVPTYVYSPAGAGFLGLAFHLQTLNDDKKQDVTEFRNSDTELLVPSFANPVPAEFLPSIFLEKDGRHDVLLSLYWRCREAKGIIVNTFEELEPYAINSLRMDSMIPPIYPVGPILNLNGEGQNSDEAAVILGWLDDQPPSSVVFLCFGSFGSFPENQVKEIAMGLERSGHRFLWSLRPCISEGETTLQLKYSNLELPAGFLDRTSCVGKVIGWAPQMAILAHEAVGGFVSHCGWNSVLESVWYGMPVATWPMYGEQQLNAFEMVKELGLAVEIEVDYRNEYNKSDFIVKADEIETKIKKLMMDGKNSKIRKKVKEMKEKSRVAMSENGSSYTSLAKLFEEIM

SEQ ID NO: 21 - DNA, 1488 bp, Barbarea vulgaris
  misc_feature: 3GT1
atggtttccgaaatcacccataaatcttatcctcttcactttgttctcttccctttcatggctcaaggccacatgattcccatggttgatattgcaaggctcttggctcagcgcggtgtgaaaataacaattgtcacaacgccgcacaatgcagcgaggttcgagaatgtcctaagccgtgccattgagtctggcttgcccatcagcatagtgcaagtcaagcttccatctcaagaagctggcttaccagaaggaaatgagactttcgattcacttgtctcaacaaagttgctggtacctttctttaaagcggttaacatgcttgaagaaccggtccagaagctctttgaagagatgagccctcaaccaagctgtataatttctgatttttgtttgccttatacaagcaaaatcgccaagaagttcaatatcccaaagatcctcttccatggcatgtgttgcttttgtcttctgtgtatgcatgttttacgcaagaaccgtgagatcttggaaaacttaaagtctgacaaggagcatttcgttgttccttattttcctgatcgagttgaattcacaagacctcaagttccattggcaacatatgttcctggggaatggcacgagatcaaggaggatatggtagaagcggataagacttcctatggtgtgatagtcaacacatatcaagagctcgagcctgcttatgccaacggctacaaggaggcaaggtctggtaaagcatggaccattggacctgtttccttgtgcaacaaggtgggagccgacaaagcagagaggggaaacaaagcagacattgatcaagatgagtgtcttaaatggcttgattctaaagaagaaggttcggttctatatgtttgccttggaagtatctgcagtcttcctctgtctcagctcaaggagctggggctaggccttgaggaatcccaaagacctttcatttgggtcgtaagaggttgggagaagaacaaagagttacttgagtggttctcggagagcggatttgaagaaagagtaaaagacagagggcttctcatcaaaggatggtcacctcaaatgcttatccttgcacatcattccgttggagggttcttaacacactgtggatggaactcgaccctcgaaggaatcacttcaggcgttccattgctcacttggccactgtttggagaccaattctgcaaccaaaaacttgtcgtgcaggtgctaaaagtgggtgtaagtgccggggttgaagaggttacgaattggggagaagaggagaaaataggagtattagtggataaagagggagtgaagaaggcagtggaagaattaatgggtgagagtgatgatgctaaagaaataagaaaaagagtcaaagagcttggacaattagctcacaaggctgtggaggaaggaggctcatctcattctaatatcacatccttgctagaagacataatgcaactagcacaacctaataattaa

SEQ ID NO: 22 - protein, 495 aa, Barbarea vulgaris
  misc_feature: 3GT1
MVSEITHKSYPLHFVLFPFMAQGHMIPMVDIARLLAQRGVKITIVTTPHNAARFENVLSRAIESGLPISIVQVKLPSQEAGLPEGNETFDSLVSTKLLVPFFKAVNMLEEPVQKLFEEMSPQPSCIISDFCLPYTSKIAKKFNIPKILFHGMCCFCLLCMHVLRKNREILENLKSDKEHFVVPYFPDRVEFTRPQVPLATYVPGEWHEIKEDMVEADKTSYGVIVNTYQELEPAYANGYKEARSGKAWTIGPVSLCNKVGADKAERGNKADIDQDECLKWLDSKEEGSVLYVCLGSICSLPLSQLKELGLGLEESQRPFIWVVRGWEKNKELLEWFSESGFEERVKDRGLLIKGWSPQMLILAHHSVGGFLTHCGWNSTLEGITSGVPLLTWPLFGDQFCNQKLVVQVLKVGVSAGVEEVTNWGEEEKIGVLVDKEGVKKAVEELMGESDDAKEIRKRVKELGQLAHKAVEEGGSSHSNITSLLEDIMQLAQPNN

SEQ ID NO: 23 - DNA, 1488 bp, Barbarea vulgaris
  misc_feature: 3GT2
atggtttccgaaatcacccataaatcttatcctcttcactttgttctcttccctttcatggctcaaggccacatgattcccatggttgatattgcaaggctcttggcccagcgcggtgtgaaaataacaattgtcacaaccccgcacaatgcagcgaggttcaagaatgtcctaagtcgtgccattgagtctggcttgcccatcagcatagtgcaagtcaagcttccatctcaagaagctggcttaccagaaggaaatgagactctcgattcacttgtctcgatggagttgatgatacatttcttaaaagcggttaacatgctggaagaaccggtccagaagctctttgaagagatgagccctcaaccaagctgtataatttctgatttttgtttgccttatacaagcaaaatcgccaagaagttcaatatcccaaagatcctcttccatggcatgtgctgcttttgtcttctgtgtatgcatattttacgcaagaaccgtgagatcgtggaaaacttaaagtctgacaaggagcatttcgttgttccttattttcctgatcgagttgaattcacaagacctcaagttccagtggcaacatatgttcctggagactggcacgagatcacggaggatatggtagaagcggataagacttcctatggtgtgatagtcaacacatatcaagagctcgagcctgcttatgccaacgactacaaggaggcaaggtctggtaaagcatggaccattggacctgtttccttgtgcaacaaggtgggagcggacaaagcagagaggggaaacaaagcagacattgatcaagatgagtgtcttaaatggcttaattctaaagaagaaggttcggttctatatgtttgccttggaagtatctgcaatcttcctctgtctcagctcaaggagctcgggctaggccttgaggaatcccaaagacctttcatttgggtcataagaggttgggagaagaacaaagagttacatgagtggttctcggagagcggattcgaagaaagaatcaaagacagaggacttctcatcaaaggatgggctcctcaaatgcttatactttcacatcattccgttggagggttcttaacacactgtggatggaactcgactcttgaggggctaaccgctggtctaccactgctgacatggccgcttttcgcagaccagttctgcaacgagaaacttgccgtgcaggtattaaaagccggtgtaagcgccggggttgaccagcctatgaaatggggagaagaggagaaaataggagtgttggtggataaagaaggagtgaagaaggcagtggaagaattaatgggtgagagtgatgatgctaaagagataagaagaagagccaaagagcttggagaattagctcacaaggctgtggaggaaggaggctcatctcattctaatatcacatcccttctagaagacataatgcaactagcacaatccaataattaa

SEQ ID NO: 24 - protein, 495 aa, Barbarea vulgaris
  misc_feature: 3GT2
MVSEITHKSYPLHFVLFPFMAQGHMIPMVDIARLLAQRGVKITIVTTPHNAARFKNVLSRAIESGLPISIVQVKLPSQEAGLPEGNETLDSLVSMELMIHFLKAVNMLEEPVQKLFEEMSPQPSCIISDFCLPYTSKIAKKFNIPKILFHGMCCFCLLCMHILRKNREIVENLKSDKEHFVVPYFPDRVEFTRPQVPVATYVPGDWHEITEDMVEADKTSYGVIVNTYQELEPAYANDYKEARSGKAWTIGPVSLCNKVGADKAERGNKADIDQDECLKWLNSKEEGSVLYVCLGSICNLPLSQLKELGLGLEESQRPFIWVIRGWEKNKELHEWFSESGFEERIKDRGLLIKGWAPQMLILSHHSVGGFLTHCGWNSTLEGLTAGLPLLTWPLFADQFCNEKLAVQVLKAGVSAGVDQPMKWGEEEKIGVLVDKEGVKKAVEELMGESDDAKEIRRRAKELGELAHKAVEEGGSSHSNITSLLEDIMQLAQSNN

SEQ ID NO: 25 - DNA, 1329 bp, Panax ginseng
  misc_feature: gGT29
atggataaccaaaaaggtagaatcagtatagcgttgctaccatttttagcccatggtcacatatctcccttctttgagctagccaaacaactcgcgaaaagaaattgcaatgttttcctctgttctaccccaatcaatcttagctccatcaaggataaggattcctctgcttctataaaactagttgagcttcatcttccatcttcccctgatcttcctcctcactatcacaccacaaatggcctcccttcccatctcatgctcccactcagaaacgcctttgaaactgcaggccccaccttctctgaaatccttaaaaccttaaaccccgatttgcttatttatgatttcaatccctcatgggcaccggagatcgcttcgtctcacaatattccggcagtttatttcctaaccacggcagcagccagctcttccattggcctacatgctttcaaaaacccaggtgaaaaatacccatttccagatttttatgataacagtaatattacccctgaaccaccttctgcagataacatgaagctacttcatgattttatcgcttgtttcgaacgatcttgcgacattattttgattaagagttttagagaactagaagggaaatatattgatttgctttccactttatctgataaaactttggttcctgttggtccactcgttcaagatcctatgggccataatgaagatccaaaaacagagcagattataaactggcttgacaaaagggctgaatctacagtggtgtttgtctgctttggaagtgagtattttctctccaatgaggaattggaagaagtagcaattgggctagagattagcacggttaatttcatatgggctgtgagattaattgaaggagagaaaaaagggattttaccagaggggtttgttcaaagggtaggagacagaggattggttgtggaggggtgggctccacaggcaagaattttaggacattcaagcaccggtgggtttgtgagccattgtgggtggagttctattgcggagagtatgaagtttggggttccagtaattgccatggccaggcatcttgatcagcctttgaatggtaagctggcggcggaggttggtgtgggcatggaggttgtgagagatgagaatgggaagtataagagagaagggattgcagaggtaataagaaaagtggttgtggagaaaagtggggaggttatcaggaggaaagcaagggagttgagtgagaaaatgaaagagaaaggagagcaagagattgatagggcattggaggagctagtacaaatttgtaagaagaagaaagatgaacaatag

SEQ ID NO: 26 - protein, 442 aa, Panax ginseng
  misc_feature: gGT29
MDNQKGRISIALLPFLAHGHISPFFELAKQLAKRNCNVFLCSTPINLSSIKDKDSSASIKLVELHLPSSPDLPPHYHTTNGLPSHLMLPLRNAFETAGPTFSEILKTLNPDLLIYDFNPSWAPEIASSHNIPAVYFLTTAAASSSIGLHAFKNPGEKYPFPDFYDNSNITPEPPSADNMKLLHDFIACFERSCDIILIKSFRELEGKYIDLLSTLSDKTLVPVGPLVQDPMGHNEDPKTEQIINWLDKRAESTVVFVCFGSEYFLSNEELEEVAIGLEISTVNFIWAVRLIEGEKKGILPEGFVQRVGDRGLVVEGWAPQARILGHSSTGGFVSHCGWSSIAESMKFGVPVIAMARHLDQPLNGKLAAEVGVGMEVVRDENGKYKREGIAEVIRKVVVEKSGEVIRRKARELSEKMKEKGEQEIDRALEELVQICKKKKDEQ

SEQ ID NO: 27 - DNA, 1329 bp, Panax ginseng
  misc_feature: gGT29-3
atggataaccaagaaggtagaatcagtatagcgttgctaccatttttagcccatggtcacatatctcccttctttgagctagccaaacaactcgcaaaaagaaattgcaatgttttcctctgttctaccccaatcaatcttagctccatcaagaataaggattcctctgcttctataaaactagttgagcttcatcttccatcttcccctgatcttcctcctcactatcacaccacaaatggcctcccttcccatctcatggtcccactcataaacgcctttgaaacagcaggccccaccttctctgaaatccttaaaaccttaaaccccgatttgcttatttatgatttcaatccctcatgggcaccggagatcgcttcgtctcacaatattccggcagtttatttcctaaccacggcagcagccagctcttccattggcctacatgctttcaaaaacccaggtgaaaaatacccatttccagatttttatgataacagtaataatacccctgaaccaccttctgcagataacatgaagctacttcatgattttatcgcttgtttcgaacgatcttgcgacattattttgattaagagttttatagaactagaagggaaatatatcgatttgctttccactttatctgataaaactttggttcctgttggtccactcgttcaagatcctatgggccataatgaagatccaaaaacagagcagattataaactggcttgacaaaagggctgaatctacagtggtgtttgtctgctttggaagtgagtattttctctccaatgaggaattggaagaagtagcaattgggctagagattagcatggttaatttcatatgggctgtgagattaattgaaggagagaaaaaaggggttttaccagagggatttgttcaaagggtaggagacagaggattggttgtggaggggtgggctccacaggcaagaattttaggacattcaagcaccggtgggtttgtgagccattgtgggtggagttctattgcggagagtatgaagtttggggttccagtaattgccatggccaggcatcttgatcagcctttgaatggtaagctggcggcggaggttggtgtgggcatggaggttgtgagagatgaaaatgggaagtataagagagaagggattgcagaggtaataagaaaagtcgttgtggagaaaagtggggaggttatgaggaggaaagcaagggaattgagtgagaaaatgaaagagaaaggagaggaagagattgatagggcagtggaggagctagtacaaatttgtaagaagaagaaagatgcacaatag

SEQ ID NO: 28 - protein, 442 aa, Panax ginseng
  misc_feature: gGT29-3
MDNQEGRISIALLPFLAHGHISPFFELAKQLAKRNCNVFLCSTPINLSSIKNKDSSASIKLVELHLPSSPDLPPHYHTTNGLPSHLMVPLINAFETAGPTFSEILKTLNPDLLIYDFNPSWAPEIASSHNIPAVYFLTTAAASSSIGLHAFKNPGEKYPFPDFYDNSNNTPEPPSADNMKLLHDFIACFERSCDIILIKSFIELEGKYIDLLSTLSDKTLVPVGPLVQDPMGHNEDPKTEQIINWLDKRAESTVVFVCFGSEYFLSNEELEEVAIGLEISMVNFIWAVRLIEGEKKGVLPEGFVQRVGDRGLVVEGWAPQARILGHSSTGGFVSHCGWSSIAESMKFGVPVIAMARHLDQPLNGKLAAEVGVGMEVVRDENGKYKREGIAEVIRKVVVEKSGEVMRRKARELSEKMKEKGEEEIDRAVEELVQICKKKKDAQ

SEQ ID NO: 29 - DNA, 20 bp, Artificial sequence
atggtttccgaaatcaccca

SEQ ID NO: 30 - DNA, 24 bp, Artificial sequence
ttaattattrgrttgtgctagttg

SEQ ID NO: 31 - DNA, 35 bp, Artificial sequence
gactggatccatggtttccgaaatcacccataaat

SEQ ID NO: 32 - DNA, 30 bp, Artificial sequence
gcgcgtcgacattattaggttgtgctagtt

SEQ ID NO: 33 - DNA, 30 bp, Artificial sequence
gcgcgtcgacattattggattgtgctagtt

SEQ ID NO: 34 - DNA, 26 bp, Artificial sequence
agtaagaaaaacagagttcatcatgg

SEQ ID NO: 35 - DNA, 20 bp, Artificial sequence
gcctcggttaggctagctgt

SEQ ID NO: 36 - DNA, 35 bp, Artificial sequence
ggcgggtaccatggataaccaaaaaggtagaatca

SEQ ID NO: 37 - DNA, 56 bp, Artificial sequence
gccgctcgagtcaatgatgatgatgatgatgttgttcatctttcttcttcttacaa

SEQ ID NO: 38 - DNA, 35 bp, Artificial sequence
ggcgggtaccatggataaccaagaaggtagaatca

SEQ ID NO: 39 - DNA, 56 bp, Artificial sequence
gccgctcgagtcaatgatgatgatgatgatgttgtgcatctttcttcttcttacaa

SEQ ID NO: 40 - DNA, 1494 bp, Medicago truncatula
  misc_feature: 3GT3
atggaaggtgttgaagttgaacaaccattgaaagtttacttcattccatttcttgcatctggacatatgatccctctttttgacatagcaactatgtttgcatcccgtggccagcaagtaacagtcatcaccactcccgccaacgcaaaatcccttaccaaatctctctcatccgacgctccttcattccttcgtcttcacaccgttgacttcccctcccaacaagtcggcctccctgaaggtattgaatctatgtcttcaactacggaccccaccaccacttggaagatccatactggcgcgatgctccttaaagaacctattggggatttcattgagaatgatccaccggattgtatcatctccgactccacgtacccatgggttaatgacttggccgataagtttcagatcccaaacatcacattcaatggattgtgcctttttgctgtctccctcgtggaaaccctcaaaacaaacaatttacttaagtctcagacagattctgattcggattcaagttcctttgttgttccaaattttcctcaccatatcaccttgtgtggaaaaccgccaaaggtaatcggtatattcatgggaatgatgcttgagacggtgcttaaaagtaaagcactaatcatcaacaacttcagtgaacttgatggagaagagtgcatacaacactacgagaaagccacgggtcacaaggtttggcatcttggtccaacttctcttattcgcaaaactgctcaagagaaatcagagaggggaaatgagggtgctgtgaatgtgcacgagagcctgagttggctcgattcagagagagttaactcagtgttgtacatatgttttggaagcatcaactatttttctgataaacaactatacgagatggcatgtgcgatagaagcatccggtcacccattcatatgggttgttcctgagaagaaagggaaagaagatgagagcgaagaagagaaagaaaagtggttaccgaagggatttgaagagagaaatatcgggaagaagggtttgatcattaggggttgggccccacaggttaagatattgagccaccctgcagtggggggatttatgacgcattgcggggggaactcaaccgtagaggctgttagtgcgggagttccaatgataacgtggccggttcatggagatcaattctacaatgagaaactgataacacaattccgaggaattggagttgaagtcggtgcaacagaatggtgtacgagtggtgtcgcggagagaaagaagttagtgagcagagatagcatagagaaggctgtaaggagattgatggacggtggtgatgaagctgaaaatatcaggctacgtgctcgagagtttggagaaaaagctatacaagctattcaagaaggtggctcgtcttataataatttgttggctttgattgacgaacttaaaagatcgagagaccttaaaagattgagagacctcaagctggatgattaa

SEQ ID NO: 41 - protein, 497 aa, Medicago truncatula
  misc_feature: 3GT3
MEGVEVEQPLKVYFIPFLASGHMIPLFDIATMFASRGQQVTVITTPANAKSLTKSLSSDAPSFLRLHTVDFPSQQVGLPEGIESMSSTTDPTTTWKIHTGAMLLKEPIGDFIENDPPDCIISDSTYPWVNDLADKFQIPNITFNGLCLFAVSLVETLKTNNLLKSQTDSDSDSSSFVVPNFPHHITLCGKPPKVIGIFMGMMLETVLKSKALIINNFSELDGEECIQHYEKATGHKVWHLGPTSLIRKTAQEKSERGNEGAVNVHESLSWLDSERVNSVLYICFGSINYFSDKQLYEMACAIEASGHPFIWVVPEKKGKEDESEEEKEKWLPKGFEERNIGKKGLIIRGWAPQVKILSHPAVGGFMTHCGGNSTVEAVSAGVPMITWPVHGDQFYNEKLITQFRGIGVEVGATEWCTSGVAERKKLVSRDSIEKAVRRLMDGGDEAENIRLRAREFGEKAIQAIQEGGSSYNNLLALIDELKRSRDLKRLRDLKLDD

SEQ ID NO: 42 - DNA, 1374 bp, Panax ginseng
  misc_feature: 3GT4
atggagagagaaatgttgagcaaaactcacattatgttcatcccattcccagctcaaggccacatgagcccaatgatgcaattcgccaagcgtttagcctggaaaggcctgcgaatcacgatagttcttccggctcaaattcgagatttcatgcaaataaccaacccattgatcaacactgagtgcatctcctttgattttgataaagacgatgggatgccatacagcatgcaggcttatatgggagttgtaaaactcaaggtcacaaataaactgagtgacctactcgagaagcaaagaacaaatggctaccctgttaatttgctagtggttgattcattatatccatctcgggtagaaatgtgccaccaacttggggtaaaaggagctccatttttcactcactcttgtgctgttggtgccatttattataatgctcgcttagggaaattgaagatacctcctgaggaagggttgacttctgtttcattgccttcaattccattgttggggagagatgatttgccaattattaggactggcacctttcctgatctctttgagcatttggggaatcagttttcagatcttgataaagcggattggatctttttcaatacttttgataagcttgaaaatgaggaagcaaaatggctatctagccaatggccaattacatccatcggaccattaatcccttcaatgtacttagacaaacaattaccaaatgacaaagacaatggcattaatttctacaaggcagacgtcggatcgtgcatcaagtggctagacgccaaagaccctggctcggtagtctacgcctcattcgggagcgtgaagcacaacctcggcgatgactacatggacgaagtagcatggggcttgttacatagcaaatatcacttcatatgggttgttatagaatccgaacgtacaaagctctctagcgatttcttggcagaggcagaggcagaggaaaaaggcctaatagtgagttggtgccctcaactccaagttttgtcacataaatctatagggagttttatgactcattgtggttggaactcgacggttgaggcattgagtttgggcgtgccaatggtggcactgccacaacagtttgatcagcctgctaatgccaagtatatcgtggatgtatggcaaattggggttcgggttccgattggtgaagagggggttgttttgaggggagaagttgctaactgtataaaggatgttatggagggggaaataggggatgagcttagagggaatgctttgaaatggaaggggttggctgtggaggcaatggagaaagggggtagctctgataagaatattgatgagttcatttcaaagcttgtttcctcctga

SEQ ID NO: 43 - protein, 457 aa, Panax ginseng
  misc_feature: 3GT4
MEREMLSKTHIMFIPFPAQGHMSPMMQFAKRLAWKGLRITIVLPAQIRDFMQITNPLINTECISFDFDKDDGMPYSMQAYMGVVKLKVTNKLSDLLEKQRTNGYPVNLLVVDSLYPSRVEMCHQLGVKGAPFFTHSCAVGAIYYNARLGKLKIPPEEGLTSVSLPSIPLLGRDDLPIIRTGTFPDLFEHLGNQFSDLDKADWIFFNTFDKLENEEAKWLSSQWPITSIGPLIPSMYLDKQLPNDKDNGINFYKADVGSCIKWLDAKDPGSVVYASFGSVKHNLGDDYMDEVAWGLLHSKYHFIWVVIESERTKLSSDFLAEAEAEEKGLIVSWCPQLQVLSHKSIGSFMTHCGWNSTVEALSLGVPMVALPQQFDQPANAKYIVDVWQIGVRVPIGEEGVVLRGEVANCIKDVMEGEIGDELRGNALKWKGLAVEAMEKGGSSDKNIDEFISKLVSS

SEQ ID NO: 44 - DNA, 24 bp, Artificial sequence
atggaaggtgttgaagttgaacaa

SEQ ID NO: 45 - DNA, 24 bp, Artificial sequence
ttaatcatccagcttgaggtctct

SEQ ID NO: 46 - DNA, 25 bp, Artificial sequence
tacataaatatataatacataggca

SEQ ID NO: 47 - DNA, 25 bp, Artificial sequence
aaaatacatacaaaatcttgaaata

SEQ ID NO: 48 - DNA, 45 bp, Artificial sequence
actttaagaaggagatataccatggaaggtgttgaagttgaacaa

SEQ ID NO: 49 - DNA, 45 bp, Artificial sequence
ctcgagtgcggccgcaagcttatcatccagcttgaggtctctcaa

SEQ ID NO: 50 - DNA, 46 bp, Artificial sequence
actttaagaaggagatataccatggagagagaaatgttgagcaaaa

SEQ ID NO: 51 - DNA, 46 bp, Artificial sequence
ctcgagtgcggccgcaagcttggaggaaacaagctttgaaatgaac

SEQ ID NO: 52 - DNA, 27 bp, Artificial sequence
ggtatatctccttcttaaagttaaaca

SEQ ID NO: 53 - DNA, 27 bp, Artificial sequence
aagcttgcggccgcactcgagcaccac

SEQ ID NO: 54 - DNA, 1341 bp, Panax ginseng
  misc_feature: gGT29-4
atggataaccaaaaaggtagaatcagtatagcgttgctaccatttttagcccatggccacatttctccattctttgagctagccaagcatctctcaaaaagaaattgtaatatattcctctgttctaccccaatcaatcttagctccatcaagaacagaatatctgataaggattcctctgcttctataaaactagtagagcttcatcttccatcttcccctgatcttcctcctcactaccacaccacaaatggcctcccttcccatctcatggtcccactcagaaacgcctttgaaacagcagcccccaccttctctgaaatccttaaaaccttaaaccctgatttgcttatttatgatttcaatccctcatgggcaccggagatcgcttcgtctcacaatattccggcagtttgtttcataattgggggagcagcctccttttccatgagcctacatagtttcaaaaacccaggtgaaaaatacccatttctagattttgatgataacagtaatattacccctgaaccaccttcagcagataacatgaagttattacttgattttatgacttgtttcgaacgatcttgcgacattattttgattaagagttttagagaactagaagggaaatattttgatttttattctactttatctgataaaactttggttcctgttggtccactcgttcaagatcctatgggccataatgaagatccaaaaacagagcagtttataaactggcttgacaaaagggctgaatctacagtggtgtttgtctgctttggaagtgagtattttctctccaatgaggaattggaagaagtagcaattgggctagagattagcatggttaatttcatatgggctgtgagattaattgaaggagagaaaaaaggggttttaccagaggggtttgttcaaagggtaggagacagaggattggttgtggaggggtgggctccacaggcaagaattttaggacattcaagcaccggtgggtttgtgagccattgtgggtggagttctattacggagagtatgaagtttggggttccagtaattgccatggccaggcatcttgatcagcctttgaatggtaagctggcggcggaggttggtgtgggcatggaggttgtgagagatgaaaatgggaagtataagagagaagggattgcagaggtaataagaaaagtcgttgtggagaaaagtggggaggttatgaggaggaaagcaagggaattgagtgagaaaatgaaagagaaaggagaggaagagattgatagggcagtggaggagctagtacaaatttgtaagaagaagaaagatgaacaatag

SEQ ID NO: 55 - protein, 446 aa, Panax ginseng
  misc_feature: gGT29-4
MDNQKGRISIALLPFLAHGHISPFFELAKHLSKRNCNIFLCSTPINLSSIKNRISDKDSSASIKLVELHLPSSPDLPPHYHTTNGLPSHLMVPLRNAFETAAPTFSEILKTLNPDLLIYDFNPSWAPEIASSHNIPAVCFIIGGAASFSMSLHSFKNPGEKYPFLDFDDNSNITPEPPSADNMKLLLDFMTCFERSCDIILIKSFRELEGKYFDFYSTLSDKTLVPVGPLVQDPMGHNEDPKTEQFINWLDKRAESTVVFVCFGSEYFLSNEELEEVAIGLEISMVNFIWAVRLIEGEKKGVLPEGFVQRVGDRGLVVEGWAPQARILGHSSTGGFVSHCGWSSITESMKFGVPVIAMARHLDQPLNGKLAAEVGVGMEVVRDENGKYKREGIAEVIRKVVVEKSGEVMRRKARELSEKMKEKGEEEIDRAVEELVQICKKKKDEQ

SEQ ID NO: 56 - DNA, 1341 bp, Panax ginseng
  misc_feature: gGT29-5
atggataaccaaaagggtagaatcagtatagttatgctgccatttttagcccatggccacatttctccattctttgagctagccaagcatctctcaaaaagaaattgtaatatattcctctgttctaccccaatcaatcttagctccatcaagaacagaatatctgataaggattcctctgcttctataaaactagtagagcttcatcttccatcttcccctgatcttcctcctcactaccacaccacaaatggcctcccttcccatctcatggtcccactcagaaacgcctttgaaacagcagcccccaccttctctgaaatccttaaaaccttaaaccctgatttgcttatttatgatttcaatccctcatgggcaccggagatcgcttcgtctcacaatattccggcagtttgtttcataattgggggagcagcctccttttccatgagcctacatagtttcaaaaacccaggtgaaaaatacccatttctagattttgatgataacagtaatattacccctgaaccaccttcagcagataacatgaagttattacttgattttatgacttgtttcgaacgatcttgcgacattattttgattaagagttttagagaactagaagggaaatatatcgatttgctttccactttatctgataaaactttggttcctgttggtccactcgttcaagatcctatgggccataatgaagatccaaaaacagagcagattataaactggcttgacaaaagggctgaatctacagtggtgtttgtctgctttggaagtgagtattttctctccaatgaggaattggaagaagtagcaattgggctagagattagcatggttaatttcatatgggctgtgagattaattgaaggagagaaaaaaggggttttaccagagggatttgttcaaagggtaggagacagaggattggttgtggaggggtgggctccacaggcaagaattttaggacattcaagcaccggtgggtttgtgagccattgtgggtggagttctattgcggagagtatgaagtttggggttccagtaattgccatggccaggcatcttgatcagcctttgaatggtaagctggcggcggaggttggtgtgggcatggaggttgtgagagatgaaaatgggaagtataagagagaagggattgcagaggtaataagaaaagtcgttgtggagaaaagtggggaggttatcaggaggaaagcaagggaattgagtgagaaaatgaaagagataggagagcaattgattgatagggcagtggaggagctagtacaaatttgtaagaagaagaaagatgaacaatag

SEQ ID NO: 57 - protein, 446 aa, Panax ginseng
  misc_feature: gGT29-5
MDNQKGRISIVMLPFLAHGHISPFFELAKHLSKRNCNIFLCSTPINLSSIKNRISDKDSSASIKLVELHLPSSPDLPPHYHTTNGLPSHLMVPLRNAFETAAPTFSEILKTLNPDLLIYDFNPSWAPEIASSHNIPAVCFIIGGAASFSMSLHSFKNPGEKYPFLDFDDNSNITPEPPSADNMKLLLDFMTCFERSCDIILIKSFRELEGKYIDLLSTLSDKTLVPVGPLVQDPMGHNEDPKTEQIINWLDKRAESTVVFVCFGSEYFLSNEELEEVAIGLEISMVNFIWAVRLIEGEKKGVLPEGFVQRVGDRGLVVEGWAPQARILGHSSTGGFVSHCGWSSIAESMKFGVPVIAMARHLDQPLNGKLAAEVGVGMEVVRDENGKYKREGIAEVIRKVVVEKSGEVIRRKARELSEKMKEIGEQLIDRAVEELVQICKKKKDEQ

SEQ ID NO: 58 - DNA, 1341 bp, Panax ginseng
  misc_feature: gGT29-6
atggataaccaaaagggtagaatcagtatagttatgctgccatttttagcccatggccacatttctccattctttgagctagccaagcatctctcaaaaagaaattgtaatatattcctctgttctaccccaatcaatcttagctccatcaagaacagaatatctgataaggattcctctgcttctataaaactagtagagcttcatcttccatcttcccctgatcttcctcctcactaccacaccacaaatggcctcccttcccatctcatggtcccactcagaaacgcctttgaaacagcagcccccaccttctctgaaatccttaaaaccttaaaccctgatttgcttatttatgatttcaatccctcatgggcaccggagatcgcttcgtctcacaatattccggcagtttatttcctaaccacggcagcagccagctcttccattggcctacatgctttcaaaaacccaggtgaaaaatacccatttccagatttttatgataacagtaataatacccctgaaccaccttctgcagataacatgaagctacttcatgattttatcgcttgtttcgaacgatcttgcgacattattttgattaagagttttatagaactagaagggaaatatatcgatttgctttccactttatctgataaaactttggttcctgttggtccactcgttcaagatcctatgggccataatgaagatccaaaaacagagcagattataaactggcttgacaaaagggctgaatctacagtggtgtttgtctgctttggaagtgagtattttctctccaatgaggaattggaagaagtagcaattgggctagagattagcatggttaatttcatatgggctgtgagattaattgaaggagagaaaaaaggggttttaccagagggatttgttcaaagggtaggagacagaggattggttgtggaggggtgggctccacaggcaagaattttaggacattcaagcaccggtgggtttgtgagccattgtgggtggagttctattgcggagagtatgaagtttggggttccagtaattgccatggccaggcatcttgatcagcctttgaatggtaagctggcggcggaggttggtgtgggcatggaggttgtgagagatgaaaatgggaagtataagagagaagatattgcaggggtaataagaaaagtcgtggtggagaaaagtggggaggttatcaggaggaaagcaagggaattgagtgagaaaatgaaagagataggagagcaattgattgatagggcagtggaggagctagtacaaatttgtaagaagaagaaagatgaacaatag

SEQ ID NO: 59 - protein, 446 aa, Panax ginseng
  misc_feature: gGT29-6
MDNQKGRISIVMLPFLAHGHISPFFELAKHLSKRNCNIFLCSTPINLSSIKNRISDKDSSASIKLVELHLPSSPDLPPHYHTTNGLPSHLMVPLRNAFETAAPTFSEILKTLNPDLLIYDFNPSWAPEIASSHNIPAVYFLTTAAASSSIGLHAFKNPGEKYPFPDFYDNSNNTPEPPSADNMKLLHDFIACFERSCDIILIKSFIELEGKYIDLLSTLSDKTLVPVGPLVQDPMGHNEDPKTEQIINWLDKRAESTVVFVCFGSEYFLSNEELEEVAIGLEISMVNFIWAVRLIEGEKKGVLPEGFVQRVGDRGLVVEGWAPQARILGHSSTGGFVSHCGWSSIAESMKFGVPVIAMARHLDQPLNGKLAAEVGVGMEVVRDENGKYKREDIAGVIRKVVVEKSGEVIRRKARELSEKMKEIGEQLIDRAVEELVQICKKKKDEQ

SEQ ID NO: 60 - DNA, 1341 bp, Panax ginseng
  misc_feature: gGT29-7
atggataaccaaaaaggtagaatcagtatagcgttgctaccatttttagcccatggtcacatatctcccttctttgagctagccaaacaactcgcaaaaagaaattgcaatgttttcctctgttctaccccaatcaatcttagctccatcaagaacagagtatctgataaggattcctctgcttctataaaactagtagagcttcatcttccatcttcccctgatcttcctcctcactaccacaccacaaatggcctcccttcccatctcatgatcccactcagaaacgcctttgatacagcaggccccaccttctctgaaatccttaaaaccttaaaccctgatttgcttatttatgatttcaatccctcatgggcaccggagatcgcttcgtctcacaatattccggcagtttgtttcataattggtggagcagcctcctcttccatgagcctacatagtttcaaaaacccaggtgaaaaatacccatttctagattttgatgataacagtaatattacccctgaaccaccttcagcagataacatgaagctattaattaattttatgacttgtttcgaacgatcttgcgacattattttgattaagagttttagagaactagaagggaaatattttgattttttttccactttatctgataaaactttggttcctgttggtccactcgttcaagatcctatgggccataatgaagatccaaaaacagagcagtttataaactggcttgacaaaagggctgaatctacagtggtgtttgtctgctttggaagtgagtgttttctctccaatgaggaattggaagaagtagcgattgggctagagattagcatggttaatttcatatgggctgtgagattaattgaaggagagaaaaaaggggttttaccagaggggtttgttcaaagggtaggagacagaggattggttgtggaggagtgggctccacaggcaagaattttaggacattcaagcaccggtgggtttgtgagccattgtgggtggaattctattacggagagtatgaagtttggggttccagtaattgccatggccaggcattttgatcagcctttgaatggtaagctggcggcggaggttggtgtgggcatggaggttgtgagagatgaaaatgggaagtataagagagaagggattgcagaggtaataagaaaagtcgttgtggagaaaagtggggaggttatcaggaggaaagcaagggaattgagtgagaaaatgaaagagaaaggagagcaagagattgatagggtagtggaggagctagtacaaatttgtaagaagaagaaagatgaacaatag

SEQ ID NO: 61 - protein, 446 aa, Panax ginseng
  misc_feature: gGT29-7
MDNQKGRISIALLPFLAHGHISPFFELAKQLAKRNCNVFLCSTPINLSSIKNRVSDKDSSASIKLVELHLPSSPDLPPHYHTTNGLPSHLMIPLRNAFDTAGPTFSEILKTLNPDLLIYDFNPSWAPEIASSHNIPAVCFIIGGAASSSMSLHSFKNPGEKYPFLDFDDNSNITPEPPSADNMKLLINFMTCFERSCDIILIKSFRELEGKYFDFFSTLSDKTLVPVGPLVQDPMGHNEDPKTEQFINWLDKRAESTVVFVCFGSECFLSNEELEEVAIGLEISMVNFIWAVRLIEGEKKGVLPEGFVQRVGDRGLVVEEWAPQARILGHSSTGGFVSHCGWNSITESMKFGVPVIAMARHFDQPLNGKLAAEVGVGMEVVRDENGKYKREGIAEVIRKVVVEKSGEVIRRKARELSEKMKEKGEQEIDRVVEELVQICKKKKDEQ

SEQ ID NO: 62 - DNA, 26 bp, Artificial sequence
acagcaagagagagacacagagttca

SEQ ID NO: 63 - DNA, 23 bp, Artificial sequence
gttcaaagcccaacctaagcgca

SEQ ID NO: 64 - DNA, 25 bp, Artificial sequence
atgaaattatacagagagggagaga

SEQ ID NO: 65 - DNA, 25 bp, Artificial sequence
tggttttcttcacaacacaaagtac

SEQ ID NO: 66 - DNA, 43 bp, Artificial sequence
ctggtgccgcgcggcagcatggataaccaaaagggtagaatca

SEQ ID NO: 67 - DNA, 43 bp, Artificial sequence
ctggtgccgcgcggcagcatggataaccaaaaaggtagaatca

SEQ ID NO: 68 - DNA, 43 bp, Artificial sequence
tgcggccgcaagcttgtcttgttcatctttcttcttcttacaa

SEQ ID NO: 69 - DNA, 30 bp, Artificial sequence
gctgccgcgcggcaccaggccgctgctgtg

SEQ ID NO: 70 - DNA, 30 bp, Artificial sequence
tccgtcgacaagcttgcggccgcactcgag